European Patent Application EP 4 442 273 A1, published October 9, 2024. Title: METHOD FOR PREVENTING AND/OR TREATING THROMBOEMBOLIC DISEASES. Applicant: SUZHOU ALPHAMAB CO., LTD. The sequence listing filed with the application follows.

SEQUENCE LISTING (350 sequences)

SEQ ID NO: 1 - protein, 123 aa, synthetic construct
  REGION 1..123: note = Artificial Sequence
QVQLQESGGGSVQAGGSLRLSCAASGYTYSFNSMGWFRQAPGKEREGVAVIYLGSTHYADSVKGRFTISQDNAKNMVYLQMNSLKPEDTAMYYCAADLLEYDGTWFGSTYNYWGQGTQVTVSS

SEQ ID NO: 2 - protein, 121 aa, synthetic construct
  REGION 1..121: note = Artificial Sequence
QVQLQESGGGLVQPGGSLRLSCAASGLTFSLYDMSWVRQAPGKGLEGVSGINSGDGSTYYADSVKGRFTISRDNAKNTLYLQMNSLKTEDTAVYYCATGRTRETYFREDDWGQGTQVTVSS

SEQ ID NO: 3 - protein, 120 aa, synthetic construct
  REGION 1..120: note = Artificial Sequence
QVQLQESGGGLVQPGGSLRLSCAASGLRFSVYDMSWVRQAPGKGLEGVSGIDSGGGSTYYADSVKGRFTISRDDAKNTLYLQMNSLKTEDTAVYYCATGLGGSWYREPDWGQGTQVTVSS

SEQ ID NO: 4 - protein, 120 aa, synthetic construct
  REGION 1..120: note = Artificial Sequence
QVQLQESGGGSVQAGGSLRLSCAGDGYTYSMGAMAWFRQAPGKEREGVALIATSSGFISYTDSVKGRFTISQDDAKIYLQMNSLKPEDTAMYYCAAGTQFSWSPGSYNYWGQGTQVTVSS

SEQ ID NO: 5 - protein, 121 aa, synthetic construct
  REGION 1..121: note = Artificial Sequence
QVQLQESGGGLVQPGGSLRLSCAASGFTFSNYDMSWVRQAPGKGLEGVSGINSGGGHPHYADSVKGRFTISRDNAKNTLYLQMNSLKTEDTAVYFCATDEGERYGEDFGYWGQGTQVTVSS

SEQ ID NO: 6 - protein, 120 aa, synthetic construct
  REGION 1..120: note = Artificial Sequence
QVQLQESGGGLVQPGGSLRVSCAASGFTFSLYDMSWVRQAPGKEREGVSGINSDDGSTSYADSVKGRFTISRDNAKNTLYLQMNSLKTEDTAVYYCATGVGARWFREDDWGQGTQVTVSS

SEQ ID NO: 7 - protein, 120 aa, synthetic construct
  REGION 1..120: note = Artificial Sequence
QVQLQESGGGLVQPGGSLRLSCAASGLRFEIYDMSWVRQAPGKGLEGVSAINSGGGSTYYADSVKGRFTISRDDVKNTLYLQMNSLKTEDTAVYYCATGDGGSWYRDGDWGQGTQVTVSS

SEQ ID NO: 8 - protein, 121 aa, synthetic construct
  REGION 1..121: note = Artificial Sequence
QVQLQESGGGLVQPGGSLRLSCVASGLTFSLYDMSWVRQAPGKGLEGVSGISGESGGSTYYADSVKGRFTISRDNAKNTLYLQMNSLKTEDTAVYYCATGDRGTWYREDDWGQGTQVTVSS

SEQ ID NO: 9 - protein, 120 aa, synthetic construct
  REGION 1..120: note = Artificial Sequence
QVQLQESGGGLVQPGGSLRLSCAASGLRFSIYDMSWVRQAPGKGLEGVSGINSGGGSTYYADSVKGRFTISRDNAKNTLYLQMNSLKTEDTAVYYCATGLGGSWFREDDWGQGTQVTVSS

SEQ ID NO: 10 - protein, 117 aa, synthetic construct
  REGION 1..117: note = Artificial Sequence
QVQLQESGGGSVQAGGSLGLSCTASGFTFDDSDMGWYRQAPGNECELVSTISSDGRGFYADSVKGRFTISQDRAKNTVYLHMNSLKPEDTAVYYCAAGWYGSFCSGLGQGTQVTVSS

SEQ ID NO: 11 - protein, 120 aa, synthetic construct
  REGION 1..120: note = Artificial Sequence
QVQLQESGGGSVQAGGSLRLSCAASGLRFSIYDWSWVRQAPGKGLEWVSAINSGGGVTSYADSVKGRVTISRDNAKNTLYLQMHSLKTEDTAVYYCATGDGGSWYRDGDWGQGTQVTVSS

SEQ ID NO: 12 - protein, 136 aa, synthetic construct
  REGION 1..136: note = Artificial Sequence
QVQLQESGGDSVQAGGSLRLSCAASGLISTGLISTRHCMSWFRQAPGKEREEVAVIGSDGSTRYGDFAKGRFTISKDTAKNTLYLQMNSLEPEDTAMYYCAAGPLVSTASRRRTRCPEGPRENIYWGQGTQVTVSS

SEQ ID NO: 13 - protein, 120 aa, synthetic construct
  REGION 1..120: note = Artificial Sequence
QVQLQESGGGLVQPGGSLRLSCAASGFTFSLYDMSWVRQAPGQGLEWVSAITNPGGSTYYADSVKDRFTISRDNAKNTLYLQMNSLKTEDTAVYYCAIGRRATFQREKDWGQGTQVTVSS

SEQ ID NO: 14 - protein, 130 aa, synthetic construct
  REGION 1..130: note = Artificial Sequence
QVQLQESGGGSVQAGGSLRLSCAASGHTYSSNYCMAWFRQAPGKEREGVAAIYSDGSTSYADSVKGRFTISKDNAKNTLYLQIDSLKPEDTSLYYCAATAYEGSWTGKQPLCLLYEYTYWGQGTQVTVSS

SEQ ID NO: 15 - protein, 119 aa, synthetic construct
  REGION 1..119: note = Artificial Sequence
QVQLQESGGGLVQPGGSLRLSCAASGFTFSLYDMSWVRQAPGKGLDGVSGIGGDGGSTYYADSVKGRFAISRDDAKNTLYLQMNSLKIEDTAVYYCALGRPPYTDYDSRGQGTQVTVSS

SEQ ID NO: 16 - protein, 124 aa, synthetic construct
  REGION 1..124: note = Artificial Sequence
QVQLQESGGGSVQAGGSLRLSCAASGFTASSNFMGWFRQAPGKEREGVAAIYTGGASTFYADSVKGRFTISQDNAKNTVYLEMDTLKPEDTAMYYCAAAPRWIAPLRADRYEYWGQGTQVTVSS

SEQ ID NO: 17 - protein, 126 aa, synthetic construct
  REGION 1..126: note = Artificial Sequence
QVQLQESGGGSVQAGGSLRLSCTASEFTFDDSDMAWYRQAPGNECELVSTITSDGGTYYADSVKGRFTISQDNAKNTMYLQMNNLKPEDTAVYYCAADQWGSAEGDCTSSYPGGYWGQGTQVTVSS

SEQ ID NO: 18 - protein, 120 aa, synthetic construct
  REGION 1..120: note = Artificial Sequence
QVQLQESGGGLVQPGGSLRLSCAASGFTFSLYDMSWVRQSPGKGLEGVSAIDSGDGRTYYADSVKGRFTISRDDAKNTLYLQMNSLKTGDTAVYYCANGGRGSWFRESDWGQGTQVTVSS

SEQ ID NO: 19 - protein, 119 aa, synthetic construct
  REGION 1..119: note = Artificial Sequence
QVQLQESGGRLVQPGGSLRLSCVASGFTFEYYDMSWVRQAPGKGLEGVSAIDARSITDYADAVKGRFTISRDNAKNTLYLQLNNLKTEDTAMYYCANGGRIGWFREDDWGQGTQVTVSS

SEQ ID NO: 20 - protein, 124 aa, synthetic construct
  REGION 1..124: note = Artificial Sequence
QVQLQESGGGSVQAGGSLRLSCVASGYTFNNNFVGWFRQAPGKEREGVAAIYSLGGSTYYADSVKGRFTISQDNAKNTVYLQMDSLKPEDTATYYCAGAITWVPPLSHRRYTYWGQGTQVTVSS

SEQ ID NO: 21 - protein, 124 aa, synthetic construct
  REGION 1..124: note = Artificial Sequence
QVQLQESGGDSVQAGGSLRLSCIASGFTFDDSDMGWYRQAPGHQCEFVSHITNDGTTYYADSVKGRFTISRDNAKNTVYLQMNSLKPEDAAVYYCAADAWGGGRSTCVNPIGYWGQGTQVTVSS

SEQ ID NO: 22 - protein, 120 aa, synthetic construct
  REGION 1..120: note = Artificial Sequence
QVQLQESGGGSVQAGGSLRLSCVASGFTGCRNIMSWYRQAPGKDREFVSAIDSDGVDYADSVKGRFSISQHNDKKTMYLQMTSLKLEDTAMYYCRRVDFGTTSQCRGNYWGQGTQVTVSS

SEQ ID NO: 23 - protein, 124 aa, synthetic construct
  REGION 1..124: note = Artificial Sequence
QVQLQESGGGSVQAGGSLRLSCAASGYTFSNNFVGWFRQAPGKKREGVATIYTLGSSTYYADSVKGRFTISQDNAKNTLYLEMNSLKPEDTAMYYCAAARGWVSPLDPARFVYWGQGTQVTVSS

SEQ ID NO: 24 - protein, 5 aa, synthetic construct
  REGION 1..5: note = Artificial Sequence
FNSMG

SEQ ID NO: 25 - protein, 14 aa, synthetic construct
  REGION 1..14: note = Artificial Sequence
IYLGSTHYADSVKG

SEQ ID NO: 26 - protein, 16 aa, synthetic construct
  REGION 1..16: note = Artificial Sequence
DLLEYDGTWFGSTYNY

SEQ ID NO: 27 - protein, 10 aa, synthetic construct
  REGION 1..10: note = Artificial Sequence
GYTYSFNSMG

SEQ ID NO: 28 - protein, 7 aa, synthetic construct
  REGION 1..7: note = Artificial Sequence
IYLGSTH

SEQ ID NO: 29 - protein, 16 aa, synthetic construct
  REGION 1..16: note = Artificial Sequence
DLLEYDGTWFGSTYNY

SEQ ID NO: 30 - protein, 7 aa, synthetic construct
  REGION 1..7: note = Artificial Sequence
GYTYSFN

SEQ ID NO: 31 - skipped

SEQ ID NO: 32 - protein, 16 aa, synthetic construct
  REGION 1..16: note = Artificial Sequence
DLLEYDGTWFGSTYNY

SEQ ID NO: 33 - protein, 8 aa, synthetic construct
  REGION 1..8: note = Artificial Sequence
GYTYSFNS

SEQ ID NO: 34 - protein, 5 aa, synthetic construct
  REGION 1..5: note = Artificial Sequence
YLGST

SEQ ID NO: 35 - protein, 18 aa, synthetic construct
  REGION 1..18: note = Artificial Sequence
AADLLEYDGTWFGSTYNY

SEQ ID NO: 36 - protein, 5 aa, synthetic construct
  REGION 1..5: note = Artificial Sequence
LYDMS

SEQ ID NO: 37 - protein, 17 aa, synthetic construct
  REGION 1..17: note = Artificial Sequence
GINSGDGSTYYADSVKG

SEQ ID NO: 38 - protein, 12 aa, synthetic construct
  REGION 1..12: note = Artificial Sequence
GRTRETYFREDD

SEQ ID NO: 39 - protein, 10 aa, synthetic construct
  REGION 1..10: note = Artificial Sequence
GLTFSLYDMS

SEQ ID NO: 40 - protein, 10 aa, synthetic construct
  REGION 1..10: note = Artificial Sequence
GINSGDGSTY

SEQ ID NO: 41 - protein, 12 aa, synthetic construct
  REGION 1..12: note = Artificial Sequence
GRTRETYFREDD

SEQ ID NO: 42 - protein, 6 aa, synthetic construct
  REGION 1..6: note = Artificial Sequence
NSGDGS

SEQ ID NO: 43 - protein, 6 aa, synthetic construct
  REGION 1..6: note = Artificial Sequence
NSGDGS

SEQ ID NO: 44 - protein, 12 aa, synthetic construct
  REGION 1..12: note = Artificial Sequence
GRTRETYFREDD

SEQ ID NO: 45 - protein, 8 aa, synthetic construct
  REGION 1..8: note = Artificial Sequence
GLTFSLYD

SEQ ID NO: 46 - protein, 8 aa, synthetic construct
  REGION 1..8: note = Artificial Sequence
INSGDGST

SEQ ID NO: 47 - protein, 14 aa, synthetic construct
  REGION 1..14: note = Artificial Sequence
ATGRTRETYFREDD

SEQ ID NO: 48 - protein, 5 aa, synthetic construct
  REGION 1..5: note = Artificial Sequence
VYDMS

SEQ ID NO: 49 - protein, 17 aa, synthetic construct
  REGION 1..17: note = Artificial Sequence
GIDSGGGSTYYADSVKG

SEQ ID NO: 50 - protein, 11 aa, synthetic construct
  REGION 1..11: note = Artificial Sequence
GLGGSWYREPD

SEQ ID NO: 51 - protein, 10 aa, synthetic construct
  REGION 1..10: note = Artificial Sequence
GLRFSVYDMS

SEQ ID NO: 52 - protein, 10 aa, synthetic construct
  REGION 1..10: note = Artificial Sequence
GIDSGGGSTY

SEQ ID NO: 53 - protein, 11 aa, synthetic construct
  REGION 1..11: note = Artificial Sequence
GLGGSWYREPD

SEQ ID NO: 54 - protein, 7 aa, synthetic construct
  REGION 1..7: note = Artificial Sequence
GLRFSVY

SEQ ID NO: 55 - protein, 6 aa, synthetic construct
  REGION 1..6: note = Artificial Sequence
DSGGGS

SEQ ID NO: 56 - protein, 11 aa, synthetic construct
  REGION 1..11: note = Artificial Sequence
GLGGSWYREPD

SEQ ID NO: 57 - protein, 8 aa, synthetic construct
  REGION 1..8: note = Artificial Sequence
GLRFSVYD

SEQ ID NO: 58 - protein, 8 aa, synthetic construct
  REGION 1..8: note = Artificial Sequence
IDSGGGST

SEQ ID NO: 59 - protein, 13 aa, synthetic construct
  REGION 1..13: note = Artificial Sequence
ATGLGGSWYREPD

SEQ ID NO: 60 - protein, 5 aa, synthetic construct
  REGION 1..5: note = Artificial Sequence
MGAMA

SEQ ID NO: 61 - protein, 17 aa, synthetic construct
  REGION 1..17: note = Artificial Sequence
LIATSSGFISYTDSVKG

SEQ ID NO: 62 - protein, 13 aa, synthetic construct
  REGION 1..13: note = Artificial Sequence
GTQFSWSPGSYNY

SEQ ID NO: 63 - protein, 10 aa, synthetic construct
  REGION 1..10: note = Artificial Sequence
GYTYSMGAMA

SEQ ID NO: 64 - protein, 10 aa, synthetic construct
  REGION 1..10: note = Artificial Sequence
LIATSSGFIS

SEQ ID NO: 65 - protein, 13 aa, synthetic construct
  REGION 1..13: note = Artificial Sequence
GTQFSWSPGSYNY

SEQ ID NO: 66 - protein, 7 aa, synthetic construct
  REGION 1..7: note = Artificial Sequence
GYTYSMG

SEQ ID NO: 67 - protein, 6 aa, synthetic construct
  REGION 1..6: note = Artificial Sequence
ATSSGF

SEQ ID NO: 68 - protein, 13 aa, synthetic construct
  REGION 1..13: note = Artificial Sequence
GTQFSWSPGSYNY

SEQ ID NO: 69 - protein, 8 aa, synthetic construct
  REGION 1..8: note = Artificial Sequence
GYTYSMGA

SEQ ID NO: 70 - protein, 8 aa, synthetic construct
  REGION 1..8: note = Artificial Sequence
IATSSGFI

SEQ ID NO: 71 - protein, 15 aa, synthetic construct
  REGION 1..15: note = Artificial Sequence
AAGTQFSWSPGSYNY

SEQ ID NO: 72 - protein, 5 aa, synthetic construct
  REGION 1..5: note = Artificial Sequence
NYDMS

SEQ ID NO: 73 - protein, 17 aa, synthetic construct
  REGION 1..17: note = Artificial Sequence
GINSGGGHPHYADSVKG

SEQ ID NO: 74 - protein, 12 aa, synthetic construct
  REGION 1..12: note = Artificial Sequence
DEGERYGEDFGY

SEQ ID NO: 75 - protein, 10 aa, synthetic construct
  REGION 1..10: note = Artificial Sequence
GFTFSNYDMS

SEQ ID NO: 76 - protein, 10 aa, synthetic construct
  REGION 1..10: note = Artificial Sequence
GINSGGGHPH

SEQ ID NO: 77 - protein, 12 aa, synthetic construct
  REGION 1..12: note = Artificial Sequence
DEGERYGEDFGY

SEQ ID NO: 78 - protein, 7 aa, synthetic construct
  REGION 1..7: note = Artificial Sequence
GFTFSNY

SEQ ID NO: 79 - protein, 6 aa, synthetic construct
  REGION 1..6: note = Artificial Sequence
NSGGGH

SEQ ID NO: 80 - protein, 12 aa, synthetic construct
  REGION 1..12: note = Artificial Sequence
DEGERYGEDFGY

SEQ ID NO: 81 - protein, 8 aa, synthetic construct
  REGION 1..8: note = Artificial Sequence
GFTFSNYD

SEQ ID NO: 82 - protein, 8 aa, synthetic construct
  REGION 1..8: note = Artificial Sequence
INSGGGHP

SEQ ID NO: 83 - protein, 14 aa, synthetic construct
  REGION 1..14: note = Artificial Sequence
ATDEGERYGEDFGY

SEQ ID NO: 84 - protein, 5 aa, synthetic construct
  REGION 1..5: note = Artificial Sequence
NYDMS

SEQ ID NO: 85 - protein, 17 aa, synthetic construct
  REGION 1..17: note = Artificial Sequence
GINSGGGHPHYADSVKG

SEQ ID NO: 86 - protein, 12 aa, synthetic construct
  REGION 1..12: note = Artificial Sequence
DEGERYGEDFGY

SEQ ID NO: 87 - protein, 10 aa, synthetic construct
  REGION 1..10: note = Artificial Sequence
GFTFSNYDMS

SEQ ID NO: 88 - protein, 10 aa, synthetic construct
  REGION 1..10: note = Artificial Sequence
GINSGGGHPH

SEQ ID NO: 89 - protein, 12 aa, synthetic construct
  REGION 1..12: note = Artificial Sequence
DEGERYGEDFGY

SEQ ID NO: 90 - protein, 7 aa, synthetic construct
  REGION 1..7: note = Artificial Sequence
GFTFSNY

SEQ ID NO: 91 - protein, 6 aa, synthetic construct
  REGION 1..6: note = Artificial Sequence
NSGGGH

SEQ ID NO: 92 - protein, 12 aa, synthetic construct
  REGION 1..12: note = Artificial Sequence
DEGERYGEDFGY

SEQ ID NO: 93 - protein, 8 aa, synthetic construct
  REGION 1..8: note = Artificial Sequence
GFTFSNYD

SEQ ID NO: 94 - protein, 8 aa, synthetic construct
  REGION 1..8: note = Artificial Sequence
INSGGGHP

SEQ ID NO: 95 - protein, 14 aa, synthetic construct
  REGION 1..14: note = Artificial Sequence
ATDEGERYGEDFGY

SEQ ID NO: 96 - protein, 5 aa, synthetic construct
  REGION 1..5: note = Artificial Sequence
IYDMS

SEQ ID NO: 97 - protein, 17 aa, synthetic construct
  REGION 1..17: note = Artificial Sequence
AINSGGGSTYYADSVKG

SEQ ID NO: 98 - protein, 11 aa, synthetic construct
  REGION 1..11: note = Artificial Sequence
GDGGSWYRDGD

SEQ ID NO: 99 - protein, 10 aa, synthetic construct
  REGION 1..10: note = Artificial Sequence
GLRFEIYDMS

SEQ ID NO: 100 - protein, 10 aa, synthetic construct
  REGION 1..10: note = Artificial Sequence
AINSGGGSTY

SEQ ID NO: 101 - protein, 11 aa, synthetic construct
  REGION 1..11: note = Artificial Sequence
GDGGSWYRDGD

SEQ ID NO: 102 - protein, 7 aa, synthetic construct
  REGION 1..7: note = Artificial Sequence
GLRFEIY

SEQ ID NO: 103 - protein, 6 aa, synthetic construct
  REGION 1..6: note = Artificial Sequence
NSGGGS

SEQ ID NO: 104 - protein, 11 aa, synthetic construct
  REGION 1..11: note = Artificial Sequence
GDGGSWYRDGD

SEQ ID NO: 105 - protein, 8 aa, synthetic construct
  REGION 1..8: note = Artificial Sequence
GLRFEIYD

SEQ ID NO: 106 - protein, 8 aa, synthetic construct
  REGION 1..8: note = Artificial Sequence
INSGGGST

SEQ ID NO: 107 - protein, 13 aa, synthetic construct
  REGION 1..13: note = Artificial Sequence
ATGDGGSWYRDGD

SEQ ID NO: 108 - protein, 5 aa, synthetic construct
  REGION 1..5: note = Artificial Sequence
LYDMS

SEQ ID NO: 109 - protein, 18 aa, synthetic construct
  REGION 1..18: note = Artificial Sequence
GISGESGGSTYYADSVKG

SEQ ID NO: 110 - protein, 11 aa, synthetic construct
  REGION 1..11: note = Artificial Sequence
GDRGTWYREDD

SEQ ID NO: 111 - protein, 10 aa, synthetic construct
  REGION 1..10: note = Artificial Sequence
GLTFSLYDMS

SEQ ID NO: 112 - protein, 11 aa, synthetic construct
  REGION 1..11: note = Artificial Sequence
GISGESGGSTY

SEQ ID NO: 113 - protein, 11 aa, synthetic construct
  REGION 1..11: note = Artificial Sequence
GDRGTWYREDD

SEQ ID NO: 114 - protein, 7 aa, synthetic construct
  REGION 1..7: note = Artificial Sequence
GLTFSLY

SEQ ID NO: 115 - protein, 7 aa, synthetic construct
  REGION 1..7: note = Artificial Sequence
SGESGGS

SEQ ID NO: 116 - protein, 11 aa, synthetic construct
  REGION 1..11: note = Artificial Sequence
GDRGTWYREDD

SEQ ID NO: 117 - protein, 8 aa, synthetic construct
  REGION 1..8: note = Artificial Sequence
GLTFSLYD

SEQ ID NO: 118 - protein, 9 aa, synthetic construct
  REGION 1..9: note = Artificial Sequence
ISGESGGST

SEQ ID NO: 119 - protein, 13 aa, synthetic construct
  REGION 1..13: note = Artificial Sequence
ATGDRGTWYREDD

SEQ ID NO: 120 - protein, 5 aa, synthetic construct
  REGION 1..5: note = Artificial Sequence
IYDMS

SEQ ID NO: 121 - protein, 17 aa, synthetic construct
  REGION 1..17: note = Artificial Sequence
GINSGGGSTYYADSVKG

SEQ ID NO: 122 - protein, 11 aa, synthetic construct
  REGION 1..11: note = Artificial Sequence
GLGGSWFREDD

SEQ ID NO: 123 - protein, 10 aa, synthetic construct
  REGION 1..10: note = Artificial Sequence
GLRFSIYDMS

SEQ ID NO: 124 - protein, 10 aa, synthetic construct
  REGION 1..10: note = Artificial Sequence
GINSGGGSTY

SEQ ID NO: 125 - protein, 11 aa, synthetic construct
  REGION 1..11: note = Artificial Sequence
GLGGSWFREDD

SEQ ID NO: 126 - protein, 7 aa, synthetic construct
  REGION 1..7: note = Artificial Sequence
GLRFSIY

SEQ ID NO: 127 - protein, 6 aa, synthetic construct
  REGION 1..6: note = Artificial Sequence
NSGGGS

SEQ ID NO: 128 - protein, 11 aa, synthetic construct
  REGION 1..11: note = Artificial Sequence
GLGGSWFREDD

SEQ ID NO: 129 - protein, 8 aa, synthetic construct
  REGION 1..8: note = Artificial Sequence
GLRFSIYD

SEQ ID NO: 130 - protein, 8 aa, synthetic construct
  REGION 1..8: note = Artificial Sequence
INSGGGST

SEQ ID NO: 131 - protein, 13 aa, synthetic construct
  REGION 1..13: note = Artificial Sequence
ATGLGGSWFREDD

SEQ ID NO: 132 - protein, 5 aa, synthetic construct
  REGION 1..5: note = Artificial Sequence
DSDMG

SEQ ID NO: 133 - protein, 16 aa, synthetic construct
  REGION 1..16: note = Artificial Sequence
TISSDGRGFYADSVKG

SEQ ID NO: 134 - protein, 9 aa, synthetic construct
  REGION 1..9: note = Artificial Sequence
GWYGSFCSG

SEQ ID NO: 135 - protein, 10 aa, synthetic construct
  REGION 1..10: note = Artificial Sequence
GFTFDDSDMG

SEQ ID NO: 136 - protein, 9 aa, synthetic construct
  REGION 1..9: note = Artificial Sequence
TISSDGRGF

SEQ ID NO: 137 - protein, 9 aa, synthetic construct
  REGION 1..9: note = Artificial Sequence
GWYGSFCSG

SEQ ID NO: 138 - protein, 7 aa, synthetic construct
  REGION 1..7: note = Artificial Sequence
GFTFDDS

SEQ ID NO: 139 - protein, 5 aa, synthetic construct
  REGION 1..5: note = Artificial Sequence
SSDGR

SEQ ID NO: 140 - protein, 9 aa, synthetic construct
  REGION 1..9: note = Artificial Sequence
GWYGSFCSG

SEQ ID NO: 141 - protein, 8 aa, synthetic construct
  REGION 1..8: note = Artificial Sequence
GFTFDDSD

SEQ ID NO: 142 - protein, 7 aa, synthetic construct
  REGION 1..7: note = Artificial Sequence
ISSDGRG

SEQ ID NO: 143 - protein, 11 aa, synthetic construct
  REGION 1..11: note = Artificial Sequence
AAGWYGSFCSG

SEQ ID NO: 144 - protein, 5 aa, synthetic construct
  REGION 1..5: note = Artificial Sequence
IYDWS

SEQ ID NO: 145 - protein, 17 aa, synthetic construct
  REGION 1..17: note = Artificial Sequence
AINSGGGVTSYADSVKG

SEQ ID NO: 146 - protein, 11 aa, synthetic construct
  REGION 1..11: note = Artificial Sequence
GDGGSWYRDGD

SEQ ID NO: 147 - protein, 10 aa, synthetic construct
  REGION 1..10: note = Artificial Sequence
GLRFSIYDWS

SEQ ID NO: 148 - protein, 10 aa, synthetic construct
  REGION 1..10: note = Artificial Sequence
AINSGGGVTS

SEQ ID NO: 149 - protein, 11 aa, synthetic construct
  REGION 1..11: note = Artificial Sequence
GDGGSWYRDGD

SEQ ID NO: 150 - protein, 7 aa, synthetic construct
  REGION 1..7: note = Artificial Sequence
GLRFSIY

SEQ ID NO: 151 - protein, 6 aa, synthetic construct
  REGION 1..6: note = Artificial Sequence
NSGGGV

SEQ ID NO: 152 - protein, 11 aa, synthetic construct
  REGION 1..11: note = Artificial Sequence
GDGGSWYRDGD

SEQ ID NO: 153 - protein, 8 aa, synthetic construct
  REGION 1..8: note = Artificial Sequence
GLRFSIYD

SEQ ID NO: 154 - protein, 8 aa, synthetic construct
  REGION 1..8: note = Artificial Sequence
GLRFSIYD

SEQ ID NO: 155 - protein, 13 aa, synthetic construct
  REGION 1..13: note = Artificial Sequence
ATGDGGSWYRDGD

SEQ ID NO: 156 - protein, 10 aa, synthetic construct
  REGION 1..10: note = Artificial Sequence
GLISTRHCMS

SEQ ID NO: 157 - protein, 16 aa, synthetic construct
  REGION 1..16: note = Artificial Sequence
VIGSDGSTRYGDFAKG

SEQ ID NO: 158 - protein, 23 aa, synthetic construct
  REGION 1..23: note = Artificial Sequence
GPLVSTASRRRTRCPEGPRENIY

SEQ ID NO: 159 - protein, 15 aa, synthetic construct
  REGION 1..15: note = Artificial Sequence
GLISTGLISTRHCMS

SEQ ID NO: 160 - protein, 9 aa, synthetic construct
  REGION 1..9: note = Artificial Sequence
VIGSDGSTR

SEQ ID NO: 161 - protein, 23 aa, synthetic construct
  REGION 1..23: note = Artificial Sequence
GPLVSTASRRRTRCPEGPRENIY

SEQ ID NO: 162 - protein, 12 aa, synthetic construct
  REGION 1..12: note = Artificial Sequence
GLISTGLISTRH

SEQ ID NO: 163 - protein, 5 aa, synthetic construct
  REGION 1..5: note = Artificial Sequence
GSDGS

SEQ ID NO: 164 - protein, 23 aa, synthetic construct
  REGION 1..23: note = Artificial Sequence
GPLVSTASRRRTRCPEGPRENIY

SEQ ID NO: 165 - protein, 13 aa, synthetic construct
  REGION 1..13: note = Artificial Sequence
GLISTGLISTRHC

SEQ ID NO: 166 - protein, 7 aa, synthetic construct
  REGION 1..7: note = Artificial Sequence
IGSDGST

SEQ ID NO: 167 - protein, 25 aa, synthetic construct
  REGION 1..25: note = Artificial Sequence
AAGPLVSTASRRRTRCPEGPRENIY

SEQ ID NO: 168 - protein, 5 aa, synthetic construct
  REGION 1..5: note = Artificial Sequence
LYDMS

SEQ ID NO: 169 - protein, 17 aa, synthetic construct
  REGION 1..17: note = Artificial Sequence
AITNPGGSTYYADSVKD

SEQ ID NO: 170 - protein, 11 aa, synthetic construct
  REGION 1..11: note = Artificial Sequence
GRRATFQREKD

SEQ ID NO: 171 - protein, 10 aa, synthetic construct
  REGION 1..10: note = Artificial Sequence
GFTFSLYDMS

SEQ ID NO: 172 - protein, 10 aa, synthetic construct
  REGION 1..10: note = Artificial Sequence
AITNPGGSTY

SEQ ID NO: 173 - protein, 11 aa, synthetic construct
  REGION 1..11: note = Artificial Sequence
GRRATFQREKD

SEQ ID NO: 174 - protein, 7 aa, synthetic construct
  REGION 1..7: note = Artificial Sequence
GFTFSLY

SEQ ID NO: 175 - protein, 6 aa, synthetic construct
  REGION 1..6: note = Artificial Sequence
TNPGGS

SEQ ID NO: 176 - protein, 11 aa, synthetic construct
  REGION 1..11: note = Artificial Sequence
GRRATFQREKD

SEQ ID NO: 177 - protein, 8 aa, synthetic construct
  REGION 1..8: note = Artificial Sequence
GFTFSLYD

SEQ ID NO: 178 - protein, 8 aa, synthetic construct
  REGION 1..8: note = Artificial Sequence
ITNPGGST

SEQ ID NO: 179 - protein, 13 aa, synthetic construct
  REGION 1..13: note = Artificial Sequence
AIGRRATFQREKD

SEQ ID NO: 180 - protein, 5 aa, synthetic construct
  REGION 1..5: note = Artificial Sequence
NYCMA

SEQ ID NO: 181 - protein, 16 aa, synthetic construct
  REGION 1..16: note = Artificial Sequence
AIYSDGSTSYADSVKG

SEQ ID NO: 182 - protein, 21 aa, synthetic construct
  REGION 1..21: note = Artificial Sequence
TAYEGSWTGKQPLCLLYEYTY

SEQ ID NO: 183 - protein, 11 aa, synthetic construct
  REGION 1..11: note = Artificial Sequence
GHTYSSNYCMA

SEQ ID NO: 184 - protein, 9 aa, synthetic construct
  REGION 1..9: note = Artificial Sequence
AIYSDGSTS

SEQ ID NO: 185 - protein, 21 aa, synthetic construct
  REGION 1..21: note = Artificial Sequence
TAYEGSWTGKQPLCLLYEYTY

SEQ ID NO: 186 - protein, 8 aa, synthetic construct
  REGION 1..8: note = Artificial Sequence
GHTYSSNY

SEQ ID NO: 187 - protein, 6 aa, synthetic construct
  REGION 1..6: note = Artificial Sequence
YSDGST

SEQ ID NO: 188 - protein, 21 aa, synthetic construct
  REGION 1..21: note = Artificial Sequence
TAYEGSWTGKQPLCLLYEYTY

SEQ ID NO: 189 - protein, 9 aa, synthetic construct
  REGION 1..9: note = Artificial Sequence
GHTYSSNYC

SEQ ID NO: 190 - protein, 7 aa, synthetic construct
  REGION 1..7: note = Artificial Sequence
IYSDGST

SEQ ID NO: 191 - protein, 23 aa, synthetic construct
  REGION 1..23: note = Artificial Sequence
AATAYEGSWTGKQPLCLLYEYTY

SEQ ID NO: 192 - protein, 5 aa, synthetic construct
  REGION 1..5: note = Artificial Sequence
LYDMS

SEQ ID NO: 193 - protein, 17 aa, synthetic construct
  REGION 1..17: note = Artificial Sequence
GIGGDGGSTYYADSVKG

SEQ ID NO: 194 - protein, 10 aa, synthetic construct
  REGION 1..10: note = Artificial Sequence
GRPPYTDYDS

SEQ ID NO: 195 - protein, 10 aa, synthetic construct
  REGION 1..10: note = Artificial Sequence
GFTFSLYDMS

SEQ ID NO: 196 - protein, 10 aa, synthetic construct
  REGION 1..10: note = Artificial Sequence
GIGGDGGSTY

SEQ ID NO: 197 - protein, 10 aa, synthetic construct
  REGION 1..10: note = Artificial Sequence
GRPPYTDYDS

SEQ ID NO: 198 - protein, 7 aa, synthetic construct
  REGION 1..7: note = Artificial Sequence
GFTFSLY

SEQ ID NO: 199 - protein, 6 aa, synthetic construct
  REGION 1..6: note = Artificial Sequence
GGDGGS

SEQ ID NO: 200 - protein, 10 aa, synthetic construct
  REGION 1..10: note = Artificial Sequence
GRPPYTDYDS

SEQ ID NO: 201 - protein, 8 aa, synthetic construct
  REGION 1..8: note = Artificial Sequence
GFTFSLYD

SEQ ID NO: 202 - protein, 8 aa, synthetic construct
  REGION 1..8: note = Artificial Sequence
IGGDGGST

SEQ ID NO: 203 - protein, 12 aa, synthetic construct
  REGION 1..12: note = Artificial Sequence
ALGRPPYTDYDS

SEQ ID NO: 204 - protein, 5 aa, synthetic construct
  REGION 1..5: note = Artificial Sequence
SNFMG

SEQ ID NO: 205 - protein, 17 aa, synthetic construct
  REGION 1..17: note = Artificial Sequence
AIYTGGASTFYADSVKG

SEQ ID NO: 206 - protein, 15 aa, synthetic construct
  REGION 1..15: note = Artificial Sequence
APRWIAPLRADRYEY

SEQ ID NO: 207 - protein, 10 aa, synthetic construct
  REGION 1..10: note = Artificial Sequence
GFTASSNFMG

SEQ ID NO: 208 - protein, 10 aa, synthetic construct
  REGION 1..10: note = Artificial Sequence
AIYTGGASTF

SEQ ID NO: 209 - protein, 15 aa, synthetic construct
  REGION 1..15: note = Artificial Sequence
APRWIAPLRADRYEY

SEQ ID NO: 210 - protein, 7 aa, synthetic construct
  REGION 1..7: note = Artificial Sequence
GFTASSN

SEQ ID NO: 211 - protein, 6 aa, synthetic construct
  REGION 1..6: note = Artificial Sequence
YTGGAS

SEQ ID NO: 212 - protein, 15 aa, synthetic construct
  REGION 1..15: note = Artificial Sequence
APRWIAPLRADRYEY

SEQ ID NO: 213 - protein, 8 aa, synthetic construct
  REGION 1..8: note = Artificial Sequence
GFTASSNF

SEQ ID NO: 214 - protein, 8 aa, synthetic construct
  REGION 1..8: note = Artificial Sequence
IYTGGAST

SEQ ID NO: 215 - protein, 17 aa, synthetic construct
  REGION 1..17: note = Artificial Sequence
AAAPRWIAPLRADRYEY

SEQ ID NO: 216 - protein, 5 aa, synthetic construct
  REGION 1..5: note = Artificial Sequence
DSDMA

SEQ ID NO: 217 - protein, 16 aa, synthetic construct
  REGION 1..16: note = Artificial Sequence
TITSDGGTYYADSVKG

SEQ ID NO: 218 - protein, 18 aa, synthetic construct
  REGION 1..18: note = Artificial Sequence
DQWGSAEGDCTSSYPGGY

SEQ ID NO: 219 - protein, 10 aa, synthetic construct
  REGION 1..10: note = Artificial Sequence
EFTFDDSDMA

SEQ ID NO: 220 - protein, 9 aa, synthetic construct
  REGION 1..9: note = Artificial Sequence
TITSDGGTY

SEQ ID NO: 221 - protein, 18 aa, synthetic construct
  REGION 1..18: note = Artificial Sequence
DQWGSAEGDCTSSYPGGY

SEQ ID NO: 222 - protein, 7 aa, synthetic construct
  REGION 1..7: note = Artificial Sequence
EFTFDDS

SEQ ID NO: 223 - protein, 5 aa, synthetic construct
  REGION 1..5: note = Artificial Sequence
TSDGG

SEQ ID NO: 224 - protein, 18 aa, synthetic construct
  REGION 1..18: note = Artificial Sequence
DQWGSAEGDCTSSYPGGY

SEQ ID NO: 225 - protein, 8 aa, synthetic construct
  REGION 1..8: note = Artificial Sequence
EFTFDDSD

SEQ ID NO: 226 - protein, 7 aa, synthetic construct
  REGION 1..7: note = Artificial Sequence
ITSDGGT

SEQ ID NO: 227 - protein, 20 aa, synthetic construct
  REGION 1..20: note = Artificial Sequence
AADQWGSAEGDCTSSYPGGY

SEQ ID NO: 228 - protein, 5 aa, synthetic construct
  REGION 1..5: note = Artificial Sequence
LYDMS

SEQ ID NO: 229 - protein, 17 aa, synthetic construct
  REGION 1..17: note = Artificial Sequence
AIDSGDGRTYYADSVKG

SEQ ID NO: 230 - protein, 11 aa, synthetic construct
  REGION 1..11: note = Artificial Sequence
GGRGSWFRESD

SEQ ID NO: 231 - protein, 10 aa, synthetic construct
  REGION 1..10: note = Artificial Sequence
GFTFSLYDMS

SEQ ID NO: 232 - protein, 10 aa, synthetic construct
  REGION 1..10: note = Artificial Sequence
AIDSGDGRTY

SEQ ID NO: 233 - protein, 11 aa, synthetic construct
  REGION 1..11: note = Artificial Sequence
GGRGSWFRESD

SEQ ID NO: 234 - protein, 7 aa, synthetic construct
  REGION 1..7: note = Artificial Sequence
GFTFSLY

SEQ ID NO: 235 - protein, 6 aa, synthetic construct
  REGION 1..6: note = Artificial Sequence
DSGDGR

SEQ ID NO: 236 - protein, 11 aa, synthetic construct
  REGION 1..11: note = Artificial Sequence
GGRGSWFRESD

SEQ ID NO: 237 - protein, 8 aa, synthetic construct
  REGION 1..8: note = Artificial Sequence
GFTFSLYD

SEQ ID NO: 238 - protein, 8 aa, synthetic construct
  REGION 1..8: note = Artificial Sequence
IDSGDGRT

SEQ ID NO: 239 - protein, 13 aa, synthetic construct
  REGION 1..13: note = Artificial Sequence
ANGGRGSWFRESD

SEQ ID NO: 240 - protein, 5 aa, synthetic construct
  REGION 1..5: note = Artificial Sequence
YYDMS

SEQ ID NO: 241 - protein, 16 aa, synthetic construct
  REGION 1..16: note = Artificial Sequence
AIDARSITDYADAVKG

SEQ ID NO: 242 - protein, 11 aa, synthetic construct
  REGION 1..11: note = Artificial Sequence
GGRIGWFREDD

SEQ ID NO: 243 - protein, 10 aa, synthetic construct
  REGION 1..10: note = Artificial Sequence
GFTFEYYDMS

SEQ ID NO: 244 - protein, 9 aa, synthetic construct
  REGION 1..9: note = Artificial Sequence
AIDARSITD

SEQ ID NO: 245 - protein, 11 aa, synthetic construct
  REGION 1..11: note = Artificial Sequence
GGRIGWFREDD

SEQ ID NO: 246 - protein, 7 aa, synthetic construct
  REGION 1..7: note = Artificial Sequence
GFTFEYY

SEQ ID NO: 247 - protein, 5 aa, synthetic construct
  REGION 1..5: note = Artificial Sequence
DARSI

SEQ ID NO: 248 - protein, 11 aa, synthetic construct
  REGION 1..11: note = Artificial Sequence
GGRIGWFREDD

SEQ ID NO: 249 - protein, 8 aa, synthetic construct
  REGION 1..8: note = Artificial Sequence
GFTFEYYD

SEQ ID NO: 250 - protein, 7 aa, synthetic construct
  REGION 1..7: note = Artificial Sequence
IDARSIT

SEQ ID NO: 251 - protein, 13 aa, synthetic construct
  REGION 1..13: note = Artificial Sequence
ANGGRIGWFREDD

SEQ ID NO: 252 - protein, 5 aa, synthetic construct
  REGION 1..5: note = Artificial Sequence
NNFVG

SEQ ID NO: 253 - protein, 17 aa, synthetic construct
  REGION 1..17: note = Artificial Sequence
AIYSLGGSTYYADSVKG

SEQ ID NO: 254 - protein, 15 aa, synthetic construct
  REGION 1..15: note = Artificial Sequence
AITWVPPLSHRRYTY

SEQ ID NO: 255 - protein, 10 aa, synthetic construct
  REGION 1..10: note = Artificial Sequence
GYTFNNNFVG

SEQ ID NO: 256 - protein, 10 aa, synthetic construct
  REGION 1..10: note = Artificial Sequence
AIYSLGGSTY

SEQ ID NO: 257 - protein, 15 aa, synthetic construct
  REGION 1..15: note = Artificial Sequence
AITWVPPLSHRRYTY

SEQ ID NO: 258 - protein, 7 aa, synthetic construct
  REGION 1..7: note = Artificial Sequence
GYTFNNN

SEQ ID NO: 259 - protein, 6 aa, synthetic construct
  REGION 1..6: note = Artificial Sequence
YSLGGS

SEQ ID NO: 260 - protein, 15 aa, synthetic construct
  REGION 1..15: note = Artificial Sequence
AITWVPPLSHRRYTY

SEQ ID NO: 261 - protein, 8 aa, synthetic construct
  REGION 1..8: note = Artificial Sequence
GYTFNNNF

SEQ ID NO: 262 - protein, 8 aa, synthetic construct
  REGION 1..8: note = Artificial Sequence
IYSLGGST

SEQ ID NO: 263 - protein, 17 aa, synthetic construct
  REGION 1..17: note = Artificial Sequence
AGAITWVPPLSHRRYTY

SEQ ID NO: 264 - protein, 5 aa, synthetic construct
  REGION 1..5: note = Artificial Sequence
DSDMG

SEQ ID NO: 265 - protein, 16 aa, synthetic construct
  REGION 1..16: note = Artificial Sequence
HITNDGTTYYADSVKG

SEQ ID NO: 266 - protein, 16 aa, synthetic construct
  REGION 1..16: note = Artificial Sequence
DAWGGGRSTCVNPIGY

SEQ ID NO: 267 - protein, 10 aa, synthetic construct
  REGION 1..10: note = Artificial Sequence
GFTFDDSDMG

SEQ ID NO: 268 - protein, 9 aa, synthetic construct
  REGION 1..9: note = Artificial Sequence
HITNDGTTY

SEQ ID NO: 269 - protein, 16 aa, synthetic construct
  REGION 1..16: note = Artificial Sequence
DAWGGGRSTCVNPIGY

SEQ ID NO: 270 - protein, 7 aa, synthetic construct
  REGION 1..7: note = Artificial Sequence
GFTFDDS

SEQ ID NO: 271 - protein, 5 aa, synthetic construct
  REGION 1..5: note = Artificial Sequence
TNDGT

SEQ ID NO: 272 - protein, 16 aa, synthetic construct
  REGION 1..16: note = Artificial Sequence
DAWGGGRSTCVNPIGY

SEQ ID NO: 273 - protein, 8 aa, synthetic construct
  REGION 1..8: note = Artificial Sequence
GFTFDDSD

SEQ ID NO: 274 - protein, 7 aa, synthetic construct
  REGION 1..7: note = Artificial Sequence
ITNDGTT

SEQ ID NO: 275 - protein, 18 aa, synthetic construct
  REGION 1..18: note = Artificial Sequence
AADAWGGGRSTCVNPIGY

SEQ ID NO: 276 - protein, 5 aa, synthetic construct
  REGION 1..5: note = Artificial Sequence
RNIMS

SEQ ID NO: 277 - protein, 15 aa, synthetic construct
  REGION 1..15: note = Artificial Sequence
AIDSDGVDYADSVKG

SEQ ID NO: 278 - protein, 13 aa, synthetic construct
  REGION 1..13: note = Artificial Sequence
VDFGTTSQCRGNY

SEQ ID NO: 279 - protein, 10 aa, synthetic construct
  REGION 1..10: note = Artificial Sequence
GFTGCRNIMS

SEQ ID NO: 280 - protein, 8 aa, synthetic construct
  REGION 1..8: note = Artificial Sequence
AIDSDGVD

SEQ ID NO: 281 - protein, 13 aa, synthetic construct
  REGION 1..13: note = Artificial Sequence
VDFGTTSQCRGNY

SEQ ID NO: 282 - protein, 7 aa, synthetic construct
  REGION 1..7: note = Artificial Sequence
GFTGCRN

SEQ ID NO: 283 - protein, 4 aa, synthetic construct
  REGION 1..4: note = Artificial Sequence
DSDG

SEQ ID NO: 284 - protein, 13 aa, synthetic construct
  REGION 1..13: note = Artificial Sequence
VDFGTTSQCRGNY

SEQ ID NO: 285 - protein, 8 aa, synthetic construct
  REGION 1..8: note = Artificial Sequence
GFTGCRNI

SEQ ID NO: 286 - protein, 6 aa, synthetic construct
  REGION 1..6: note = Artificial Sequence
IDSDGV

SEQ ID NO: 287 - protein, 15 aa, synthetic construct
  REGION 1..15: note = Artificial Sequence
RRVDFGTTSQCRGNY

SEQ ID NO: 288 - protein, 5 aa, synthetic construct
  REGION 1..5: note = Artificial Sequence
NNFVG

SEQ ID NO: 289 - protein, 17 aa, synthetic construct
  REGION 1..17: note = Artificial Sequence
TIYTLGSSTYYADSVKG

SEQ ID NO: 290 - protein, 15 aa, synthetic construct
  REGION 1..15: note = Artificial Sequence
ARGWVSPLDPARFVY

SEQ ID NO: 291 - protein, 10 aa, synthetic construct
  REGION 1..10: note = Artificial Sequence
GYTFSNNFVG

SEQ ID NO: 292 - protein, 10 aa, synthetic construct
  REGION 1..10: note = Artificial Sequence
TIYTLGSSTY

SEQ ID NO: 293 - protein, 15 aa, synthetic construct
  REGION 1..15: note = Artificial Sequence
ARGWVSPLDPARFVY

SEQ ID NO: 294 - protein, 7 aa, synthetic construct
  REGION 1..7: note = Artificial Sequence
GYTFSNN

SEQ ID NO: 295 - protein, 6 aa, synthetic construct
  REGION 1..6: note = Artificial Sequence
YTLGSS

SEQ ID NO: 296 - protein, 15 aa, synthetic construct
  REGION 1..15: note = Artificial Sequence
ARGWVSPLDPARFVY

SEQ ID NO: 297 - protein, 8 aa, synthetic construct
  REGION 1..8: note = Artificial Sequence
GYTFSNNF

SEQ ID NO: 298 - protein, 8 aa, synthetic construct
  REGION 1..8: note = Artificial Sequence
IYTLGSST

SEQ ID NO: 299 - protein, 17 aa, synthetic construct
  REGION 1..17: note = Artificial Sequence
AAARGWVSPLDPARFVY

SEQ ID NO: 300 - protein, 123 aa, synthetic construct
  REGION 1..123: note = Artificial Sequence
QVQLVESGGGSVQAGGSLRLSCAASGYTYSFNSMGWFRQAPGKEREGVAVIYLGSTHYADSVKGRFTISQDNSKNTVYLQMNSLRAEDTAVYYCAADLLEYDGTWFGSTYNYWGQGTLVTVSS

SEQ ID NO: 301 - protein, 123 aa, synthetic construct
  REGION 1..123: note = Artificial Sequence
QVQLVESGGGLVQPGGSLRLSCAASGYTYSFNSMGWFRQAPGKGLEGVSVIYLGSTHYADSVKGRFTISRDNSKNTLYLQMNSLRAEDTAVYYCAADLLEYDGTWFGSTYNYWGQGTLVTVSS

SEQ ID NO: 302 - protein, 123 aa, synthetic construct
  REGION 1..123: note = Artificial Sequence
QVQLVESGGGLVQPGGSLRLSCAASGYTYSFNSMGWFRQAPGKEREGVAVIYLGSTHYADSVKGRFTISQDNSKNTVYLQMNSLRAEDTAVYYCAADLLEYDGTWFGSTYNYWGQGTLVTVSS

SEQ ID NO: 303 - protein, 123 aa, synthetic construct
  REGION 1..123: note = Artificial Sequence
QVQLVESGGGSVQAGGSLRLSCAASGYTYSFNSMGWFRQAPGKGLEGVSVIYLGSTHYADSVKGRFTISQDNSKNTVYLQMNSLRAEDTAVYYCAADLLEYDGTWFGSTYNYWGQGTLVTVSS

SEQ ID NO: 304 - protein, 123 aa, synthetic construct
  REGION 1..123: note = Artificial Sequence
QVQLVESGGGSVQAGGSLRLSCAASGYTYSFNSMGWFRQAPGKGLEGVSVIYLGSTHYADSVKGRFTISQDNSKNTLYLQMNSLKPEDTAVYYCAADLLEYDGTWFGSTYNYWGQGTLVTVSS

SEQ ID NO: 305 - protein, 123 aa, synthetic construct
  REGION 1..123: note = Artificial Sequence
QVQLVESGGGLVQPGGSLRLSCAASGYTYSFNSMGWFRQAPGKGLEGVSVIYLGSTHYADSVKGRFTISQDNSKNTLYLQMNSLKPEDTAVYYCAADLLEYDGTWFGSTYNYWGQGTLVTVSS

SEQ ID NO: 306 - protein, 122 aa, synthetic construct
  REGION 1..122: note = Artificial Sequence
QVQLVESGGGSVQAGGSLRLSCAASGYTYSMGAMAWFRQAPGKEREGVALIATSSGFISYTDSVKGRFTISQDNSKNTVYLQMNSLRAEDTAVYYCAAGTQFSWSPGSYNYWGQGTLVTVSS

SEQ ID NO: 307 - protein, 122 aa, synthetic construct
  REGION 1..122: note = Artificial Sequence
QVQLVESGGGLVQPGGSLRLSCAASGYTYSMGAMAWFRQAPGKGLEGVSLIATSSGFISYTDSVKGRFTISRDNSKNTLYLQMNSLRAEDTAVYYCAAGTQFSWSPGSYNYWGQGTLVTVSS

SEQ ID NO: 308 - protein, 122 aa, synthetic construct
  REGION 1..122: note = Artificial Sequence
QVQLVESGGGLVQPGGSLRLSCAASGYTYSMGAMAWFRQAPGKEREGVALIATSSGFISYTDSVKGRFTISQDNSKNTVYLQMNSLRAEDTAVYYCAAGTQFSWSPGSYNYWGQGTLVTVSS

SEQ ID NO: 309 - protein, 122 aa, synthetic construct
  REGION 1..122: note = Artificial Sequence
QVQLVESGGGSVQAGGSLRLSCAASGYTYSMGAMAWFRQAPGKGLEGVSLIATSSGFISYTDSVKGRFTISQDNSKNTVYLQMNSLRAEDTAVYYCAAGTQFSWSPGSYNYWGQGTLVTVSS

SEQ ID NO: 310 - protein, 122 aa, synthetic construct
  REGION 1..122: note = Artificial Sequence
QVQLVESGGGSVQAGGSLRLSCAASGYTYSMGAMAWFRQAPGKGLEGVSLIATSSGFISYTDSVKGRFTISQDNSKNTLYLQMNSLKPEDTAVYYCAAGTQFSWSPGSYNYWGQGTLVTVSS

SEQ ID NO: 311 - protein, 122 aa, synthetic construct
  REGION 1..122: note = Artificial Sequence
QVQLVESGGGLVQPGGSLRLSCAASGYTYSMGAMAWFRQAPGKGLEGVSLIATSSGFISYTDSVKGRFTISQDNSKNTLYLQMNSLKPEDTAVYYCAAGTQFSWSPGSYNYWGQGTLVTVSS

SEQ ID NO: 312 - protein, 117 aa, synthetic construct
  REGION 1..117: note = Artificial Sequence
QVQLVESGGGSVQAGGSLRLSCTASGFTFDDSDMGWYRQAPGNECELVSTISSDGRGFYADSVKGRFTISQDNSKNTVYLQMNSLRAEDTAVYYCAAGWYGSFCSGLGQGTLVTVSS

SEQ ID NO: 313 - protein, 117 aa, synthetic construct
  REGION 1..117: note = Artificial Sequence
QVQLVESGGGLVQPGGSLRLSCAASGFTFDDSDMGWYRQAPGNECELVSTISSDGRGFYADSVKGRFTISRDNSKNTLYLQMNSLRAEDTAVYYCAAGWYGSFCSGLGQGTLVTVSS

SEQ ID NO: 314 - protein, 117 aa, synthetic construct
  REGION 1..117: note = Artificial Sequence
QVQLVESGGGLVQPGGSLRLSCTASGFTFDDSDMGWYRQAPGNECELVSTISSDGRGFYADSVKGRFTISRDNSKNTVYLQMNSLRAEDTAVYYCAAGWYGSFCSGLGQGTLVTVSS

SEQ ID NO: 315 - protein, 117 aa, synthetic construct; identical to SEQ ID NO: 312
  REGION 1..117: note = Artificial Sequence

SEQ ID NO: 316 - protein, 117 aa, synthetic construct
  REGION 1..117: note = Artificial Sequence
QVQLVESGGGSVQAGGSLRLSCTASGFTFDDSDMGWYRQAPGNECELVSTISSDGRGFYADSVKGRFTISQDNSKNTLYLQMNSLKPEDTAVYYCAAGWYGSFCSGLGQGTLVTVSS

SEQ ID NO: 317 - protein, 117 aa, synthetic construct
  REGION 1..117: note = Artificial Sequence
QVQLVESGGGLVQPGGSLRLSCTASGFTFDDSDMGWYRQAPGNECELVSTISSDGRGFYADSVKGRFTISRDNSKNTLYLQMNSLKPEDTAVYYCAAGWYGSFCSGLGQGTLVTVSS

SEQ ID NO: 318 - protein, 130 aa, synthetic construct
  REGION 1..130: note = Artificial Sequence
QVQLVESGGGSVQAGGSLRLSCAASGHTYSSNYCMAWFRQAPGKEREGVAAIYSDGSTSYADSVKGRFTISKDNSKNTLYLQMNSLRAEDTAVYYCAATAYEGSWTGKQPLCLLYEYTYWGQGTLVTVSS

SEQ ID NO: 319 - protein, 130 aa, synthetic construct
  REGION 1..130: note = Artificial Sequence
QVQLVESGGGLVQPGGSLRLSCAASGHTYSSNYCMAWFRQAPGKEREGVAAIYSDGSTSYADSVKGRFTISRDNSKNTLYLQMNSLRAEDTAVYYCAATAYEGSWTGKQPLCLLYEYTYWGQGTLVTVSS

SEQ ID NO: 320 - protein, 130 aa, synthetic construct
  REGION 1..130: note = Artificial Sequence
QVQLVESGGGLVQPGGSLRLSCAASGHTYSSNYCMAWFRQAPGKEREGVAAIYSDGSTSYADSVKGRFTISKDNSKNTLYLQMNSLRAEDTAVYYCAATAYEGSWTGKQPLCLLYEYTYWGQGTLVTVSS

SEQ ID NO: 321 - protein, 130 aa, synthetic construct
  REGION 1..130: note = Artificial Sequence
QVQLVESGGGSVQAGGSLRLSCAASGHTYSSNYCMAWFRQAPGKGLEGVSAIYSDGSTSYADSVKGRFTISKDNSKNTLYLQMNSLRAEDTAVYYCAATAYEGSWTGKQPLCLLYEYTYWGQGTLVTVSS

SEQ ID NO: 322 - protein, 130 aa, synthetic construct
  REGION 1..130: note = Artificial Sequence
QVQLVESGGGSVQAGGSLRLSCAASGHTYSSNYCMAWFRQAPGKGLEGVSAIYSDGSTSYADSVKGRFTISKDNSKNTLYLQMNSLKPEDTAVYYCAATAYEGSWTGKQPLCLLYEYTYWGQGTLVTVSS

SEQ ID NO: 323 - protein, 130 aa, synthetic construct
  REGION 1..130: note = Artificial Sequence
QVQLVESGGGLVQPGGSLRLSCAASGHTYSSNYCMAWFRQAPGKGLEGVSAIYSDGSTSYADSVKGRFTISKDNSKNTLYLQMNSLKPEDTAVYYCAATAYEGSWTGKQPLCLLYEYTYWGQGTLVTVSS

SEQ ID NO: 324 - protein, 126 aa, synthetic construct
  REGION 1..126: note = Artificial Sequence
QVQLVESGGGSVQAGGSLRLSCTASEFTFDDSDMAWYRQAPGNECELVSTITSDGGTYYADSVKGRFTISQDNSKNTMYLQMNSLRAEDTAVYYCAADQWGSAEGDCTSSYPGGYWGQGTLVTVSS

SEQ ID NO: 325 - protein, 126 aa, synthetic construct
  REGION 1..126: note = Artificial Sequence
QVQLVESGGGLVQPGGSLRLSCAASEFTFDDSDMAWYRQAPGNECELVSTITSDGGTYYADSVKGRFTISRDNSKNTLYLQMNSLRAEDTAVYYCAADQWGSAEGDCTSSYPGGYWGQGTLVTVSS

SEQ ID NO: 326 - protein, 126 aa, synthetic construct
  REGION 1..126: note = Artificial Sequence
QVQLVESGGGLVQPGGSLRLSCTASEFTFDDSDMAWYRQAPGNECELVSTITSDGGTYYADSVKGRFTISQDNSKNTMYLQMNSLRAEDTAVYYCAADQWGSAEGDCTSSYPGGYWGQGTLVTVSS

SEQ ID NO: 327 - protein, 126 aa, synthetic construct
  REGION 1..126: note = Artificial Sequence
QVQLVESGGGSVQAGGSLRLSCTASEFTFDDSDMAWYRQAPGNECELVSTITSDGGTYYADSVKGRFTISRDNSKNTMYLQMNSLRAEDTAVYYCAADQWGSAEGDCTSSYPGGYWGQGTLVTVSS

SEQ ID NO: 328 - protein, 126 aa, synthetic construct
  REGION 1..126: note = Artificial Sequence
QVQLVESGGGSVQAGGSLRLSCTASEFTFDDSDMAWYRQAPGNECELVSTITSDGGTYYADSVKGRFTISRDNSKNTLYLQMNSLKPEDTAVYYCAADQWGSAEGDCTSSYPGGYWGQGTLVTVSS

SEQ ID NO: 329 - protein, 126 aa, synthetic construct
  REGION 1..126: note = Artificial Sequence
QVQLVESGGGLVQPGGSLRLSCTASEFTFDDSDMAWYRQAPGNECELVSTITSDGGTYYADSVKGRFTISRDNSKNTLYLQMNSLKPEDTAVYYCAADQWGSAEGDCTSSYPGGYWGQGTLVTVSS

SEQ ID NO: 330 - protein, 124 aa, synthetic construct
  REGION 1..124: note = Artificial Sequence
QVQLVESGGGSVQAGGSLRLSCAASGYTFNNNFVGWFRQAPGKEREGVAAIYSLGGSTYYADSVKGRFTISQDNSKNTVYLQMNSLRAEDTAVYYCAGAITWVPPLSHRRYTYWGQGTLVTVSS

SEQ ID NO: 331 - protein, 124 aa, synthetic construct
  REGION 1..124: note = Artificial Sequence
QVQLVESGGGLVQPGGSLRLSCAASGYTFNNNFVGWFRQAPGKGLEGVSAIYSLGGSTYYADSVKGRFTISRDNSKNTLYLQMNSLRAEDTAVYYCAAAITWVPPLSHRRYTYWGQGTLVTVSS

SEQ ID NO: 332 - protein, 124 aa, synthetic construct
  REGION 1..124: note = Artificial Sequence
QVQLVESGGGLVQPGGSLRLSCAASGYTFNNNFVGWFRQAPGKEREGVAAIYSLGGSTYYADSVKGRFTISQDNSKNTVYLQMNSLRAEDTAVYYCAGAITWVPPLSHRRYTYWGQGTLVTVSS

SEQ ID NO: 333 - protein, 124 aa, synthetic construct
  REGION 1..124: note = Artificial Sequence
QVQLVESGGGSVQAGGSLRLSCAASGYTFNNNFVGWFRQAPGKGLEGVSAIYSLGGSTYYADSVKGRFTISQDNSKNTVYLQMNSLRAEDTAVYYCAGAITWVPPLSHRRYTYWGQGTLVTVSS

SEQ ID NO: 334 - protein, 124 aa, synthetic construct
  REGION 1..124: note = Artificial Sequence
QVQLVESGGGSVQAGGSLRLSCAASGYTFNNNFVGWFRQAPGKGLEGVSAIYSLGGSTYYADSVKGRFTISQDNSKNTLYLQMNSLKPEDTAVYYCAGAITWVPPLSHRRYTYWGQGTLVTVSS

SEQ ID NO: 335 - protein, 124 aa, synthetic construct
  REGION 1..124: note = Artificial Sequence
QVQLVESGGGSVQAGGSLRLSCAASGYTFNNNFVGWFRQAPGKGLEGVSAIYSLGGSTYYADSVKGRFTISRDNSKNTLYLQMNSLKPEDTAVYYCAGAITWVPPLSHRRYTYWGQGTLVTVSS

SEQ ID NO: 336 - protein, 232 aa, synthetic construct
  REGION 1..232: note = Artificial Sequence
EPKSCDKTHTCPPCPAPELLGGPSVFLFPPKPKDTLMISRTPEVTCVVVDVSHEDPEVKFNWYVDGVEVHNAKTKPREEQYNSTYRVVSVLTVLHQDWLNGKEYKCKVSNKALPAPIEKTISKAKGQPREPQVYTLPPSRDELTKNQVSLTCLVKGFYPSDIAVEWESNGQPENNYKTTPPVLDSDGSFFLYSKLTVDKSRWQQGNVFSCSVMHEALHNHYTQKSLSLSPGK

SEQ ID NO: 337 - protein, 91 aa, synthetic construct
  REGION 1..91: note = Artificial Sequence
ECVTQLLKDTCFEGGDITTVFTPSAKYCQVVCTYHPRCLLFTFTAESPSEDPTRWFTCVLKDSVTETLPRVNRTAAISGYSFKQCSHQISA

SEQ ID NO: 338 - protein, 95 aa, synthetic construct
  REGION 1..95: note = Artificial Sequence
HQISACNKDIYVDLDMKGINYNSSVAKSAQECQERCTDDVHCHFFTYATRQFPSLEHRNICLLKHTQTGTPTRITKLDKVVSGFSLKSCALSNLA

SEQ ID NO: 339 - protein, 96 aa, synthetic construct
  REGION 1..96: note = Artificial Sequence
LSNLACIRDIFPNTVFADSNIDSVMAPDAFVCGRICTHHPGCLFFTFFSQEWPKESQRNLCLLKTSESGLPSTRIKKSKALSGFSLQSCRHSIPVF

SEQ ID NO: 340 - protein, 97 aa, synthetic construct
  REGION 1..97: note = Artificial Sequence
IPVFCHSSFYHDTDFLGEELDIVAAKSHEACQKLCTNAVRCQFFTYTPAQASCNEGKGKCYLKLSSNGSPTKILHGRGGISGYTLRLCKMDNESTTK

SEQ ID NO: 341 - protein, 181 aa, synthetic construct
  REGION 1..181: note = Artificial Sequence
ECVTQLLKDTCFEGGDITTVFTPSAKYCQVVCTYHPRCLLFTFTAESPSEDPTRWFTCVLKDSVTETLPRVNRTAAISGYSFKQCSHQISACNKDIYVDLDMKGINYNSSVAKSAQECQERCTDDVHCHFFTYATRQFPSLEHRNICLLKHTQTGTPTRITKLDKVVSGFSLKSCALSNLA

SEQ ID NO: 342 - protein, 186 aa, synthetic construct
  REGION 1..186: note = Artificial Sequence
HQISACNKDIYVDLDMKGINYNSSVAKSAQECQERCTDDVHCHFFTYATRQFPSLEHRNICLLKHTQTGTPTRITKLDKVVSGFSLKSCALSNLACIRDIFPNTVFADSNIDSVMAPDAFVCGRICTHHPGCLFFTFFSQEWPKESQRNLCLLKTSESGLPSTRIKKSKALSGFSLQSCRHSIPVF

SEQ ID NO: 343 - protein, 186 aa, synthetic construct; identical to SEQ ID NO: 342
  REGION 1..186: note = Artificial Sequence

SEQ ID NO: 344 - protein, 493 aa, synthetic construct
  REGION 1..493: note = KN060 single chain
QVQLVESGGGSVQAGGSLRLSCAASGHTYSSNYCMAWFRQAPGKEREGVAAIYSDGSTSYADSVKGRFTISKDNSKNTLYLQMNSLRAEDTAVYYCAATAYEGSWTGKQPLCLLYEYTYWGQGTLVTVSSGAPQVQLVESGGGSVQAGGSLRLSCTASEFTFDDSDMAWYRQAPGNECELVSTITSDGGTYYADSVKGRFTISQDNSKNTMYLQMNSLRAEDTAVYYCAADQWGSAEGDCTSSYPGGYWGQGTLVTVSSGSEPKSSDKTHTCPPCPAPELLGGPSVFLFPPKPKDTLMISRTPEVTCVVVDVSHEDPEVKFNWYVDGVEVHNAKTKPREEQYNSTYRVVSVLTVLHQDWLNGKEYKCKVSNKALPAPIEKTISKAKGQPREPQVYTLPPSRDELTKNQVSLTCLVKGFYPSDIAVEWESNGQPENNYKTTPPVLDSDGSFFLYSKLTVDKSRWQQGNVFSCSVMHEALHNHYTQKSLSLSPGK

SEQ ID NO: 345 - protein, 446 aa, synthetic construct
  REGION 1..446: note = 14E11 heavy chain
QVQLEESGPGLVAPSQSLSITCTVSGFSLTGYGIYWVRQPPGKGLEWLGMIWGDGRTDYNSALKSRLSISKDNSKSQVFLKMNSLQTDDTARYYCARDYYGSKDYWGQGTTLTVSSASTKGPSVFPLAPSSKSTSGGTAALGCLVKDYFPEPVTVSWNSGALTSGVHTFPAVLQSSGLYSLSSVVTVPSSSLGTQTYICNVNHKPSNTKVDKKVEPKSCDKTHTCPPCPAPELLGGPSVFLFPPKPKDTLMISRTPEVTCVVVDVSHEDPEVKFNWYVDGVEVHNAKTKPREEQYNSTYRVVSVLTVLHQDWLNGKEYKCKVSNKALPAPIEKTISKAKGQPREPQVYTLPPSRDELTKNQVSLTCLVKGFYPSDIAVEWESNGQPENNYKTTPPVLDSDGSFFLYSKLTVDKSRWQQGNVFSCSVMHEALHNHYTQKSLSLSPGK

SEQ ID NO: 346 - protein, 215 aa, synthetic construct
  REGION 1..215: note = 14E11 light chain
DIVMTQSHKFMSTSVGDRVSITCKASQDVSTAVAWYQQKPGQSPKLLIYLTSYRNTGVPDRFTGSGSGTDFTFTISSVQAEDLAVYYCQQHYKTPYSFGGGTKLERLRRTVAAPSVFIFPPSDEQLKSGTASVVCLLNNFYPREAKVQWKVDNALQSGNSQESVTEQDSKDSTYSLSSTLTLSKADYEKHKVYACEVTHQGLSSPVTKSFNRGEC

SEQ ID NO: 347 - protein, 449 aa, synthetic construct
  REGION 1..449: note = BAY1213790 heavy chain
EVQLLESGGGLVQPGGSLRLSCAASGFTFSQYGMDWVRQAPGKGLEWVSGIGPSGGSTVYADSVKGRFTISRDNSKNTLYLQMNSLRAEDTAVYYCTRGGPYYYYGMDVWGQGTTVTVSSASTKGPSVFPLAPSSKSTSGGTAALGCLVKDYFPEPVTVSWNSGALTSGVHTFPAVLQSSGLYSLSSVVTVPSSSLGTQTYICNVNHKPSNTKVDKKVEPKSCDKTHTCPPCPAPELLGGPSVFLFPPKPKDTLMISRTPEVTCVVVDVSHEDPEVKFNWYVDGVEVHNAKTKPREEQYNSTYRVVSVLTVLHQDWLNGKEYKCKVSNKALPAPIEKTISKAKGQPREPQVYTLPPSRDELTKNQVSLTCLVKGFYPSDIAVEWESNGQPENNYKTTPPVLDSDGSFFLYSKLTVDKSRWQQGNVFSCSVMHEALHNHYTQKSLSLSPG

SEQ ID NO: 348 - protein, 214 aa, synthetic construct
  REGION 1..214: note = BAY1213790 light chain
DIQMTQSPSSLSASVGDRVTITCQASQDISNYLNWYQQKPGKAPKLLIYDASNLETGVPSRFSGSGSGTDFTFTISSLQPEDIATYYCQQADSFPVTFGGGTKVEIKRTVAAPSVFIFPPSDEQLKSGTASVVCLLNNFYPREAKVQWKVDNALQSGNSQESVTEQDSKDSTYSLSSTLTLSKADYEKHKVYACEVTHQGLSSPVTKSFNRGEC

SEQ ID NO: 349 - protein, 130 aa, synthetic construct; identical to SEQ ID NO: 318
  REGION 1..130: note = KN060 VH

SEQ ID NO: 350 - protein, 126 aa, synthetic construct; identical to SEQ ID NO: 324
  REGION 1..126: note = KN060 VHH